European Patent Specification EP 3 692 051 B9, published October 4, 2023. Title: ANTICANCER PEPTIDES AND USES THEREOF. Applicant: Suigeneris Farmacosmetics S.L. The sequence listing filed with the application follows.

SEQUENCE LISTING (6 sequences)

SEQ ID NO: 1 - protein, 7 aa, Artificial
  PEPTIDE
  MOD_RES (7)..(7): AMIDATION
CFEISKY

SEQ ID NO: 2 - protein, 7 aa, Artificial
  PEPTIDE
  MOD_RES (1)..(1): ACETYLATION
  MOD_RES (7)..(7): AMIDATION
CFEVSKY

SEQ ID NO: 3 - protein, 7 aa, Artificial
  PEPTIDE
  MOD_RES (1)..(1): ACETYLATION
  MOD_RES (7)..(7): AMIDATION
CFEISKY

SEQ ID NO: 4 - protein, 6 aa, Artificial
  PEPTIDE
  MOD_RES (1)..(1): ACETYLATION
  MOD_RES (6)..(6): AMIDATION
FEISKY

SEQ ID NO: 5 - protein, 6 aa, Artificial
  PEPTIDE
  MOD_RES (1)..(1): ACETYLATION
  MOD_RES (6)..(6): AMIDATION
VFSTAL

SEQ ID NO: 6 - protein, 7 aa, Artificial
  PEPTIDE
  MOD_RES (1)..(1): ACETYLATION
  MOD_RES (6)..(6): AMIDATION
CVFSTAL